European Patent Specification EP 4 041 763 B1, published February 26, 2025. Title: PD1 AND VEGFR2 DUAL-BINDING AGENTS. Applicant: ULTRAHUMAN EIGHT LIMITED. The sequence listing filed with the application follows.

SEQUENCE LISTING (75 sequences)

SEQ ID NO: 1 - protein, 10 aa, Artificial Sequence
  VH HCDR1
GFTFSSYMMS

SEQ ID NO: 2 - protein, 17 aa, Artificial Sequence
  VH HCDR2
TISGGGANTYYPDSVKG

SEQ ID NO: 3 - protein, 7 aa, Artificial Sequence
  VH HCDR3
QLYYFDY

SEQ ID NO: 4 - protein, 11 aa, Artificial Sequence
  VL LCDR1
LASQGIGPWLS

SEQ ID NO: 5 - protein, 7 aa, Artificial Sequence
  VL LCDR2
TATSLAD

SEQ ID NO: 6 - protein, 9 aa, Artificial Sequence
  VL LCDR3
QQVYSIPWT

SEQ ID NO: 7 - protein, 11 aa, Artificial Sequence
  VL LCDR1
LASQPLGIWLS

SEQ ID NO: 8 - protein, 11 aa, Artificial Sequence
  VL LCDR1
LASQESGIWLS

SEQ ID NO: 9 - protein, 11 aa, Artificial Sequence
  VL LCDR1
LASQTIGTWLT

SEQ ID NO: 10 - protein, 9 aa, Artificial Sequence
  VL LCDR3
QQVAELPFG

SEQ ID NO: 11 - protein, 9 aa, Artificial Sequence
  VL LCDR3
QQVSVTPFT

SEQ ID NO: 12 - protein, 11 aa, Artificial Sequence
  VL LCDR1
LASQESGIWLG

SEQ ID NO: 13 - protein, 116 aa, Artificial Sequence
  heavy chain variable (VH) region
EVQLVESGGGLVQPGGSLRLSCAASGFTFSSYMMSWVRQAPGKGLEWVATISGGGANTYYPDSVKGRFTISRDNAKNSLYLQMNSLRAEDTAVYYCARQLYYFDYWGQGTTVTVSS

SEQ ID NO: 14 - protein, 107 aa, Artificial Sequence
  light chain variable (VL) region
DIQMTQSSSSLSASVGDRVTITCLASQGIGPWLSWYQQKPGKAPKLLIYTATSLADGVPSRFSGSGSGTDFTLTISSLQPEDFATYYCQQVYSIPWTFGGGTKVEIK

SEQ ID NO: 15 - protein, 107 aa, Artificial Sequence
  light chain variable (VL) region
DIQMTQSPSSLSASVGDRVTITCLASQPLGIWLSWYQQKPGKAPKLLIYTATSLADGVPSRFSGSGSGTDFTLTISSLQPEDFATYYCQQVYSIPWTFGGGTKVEIK

SEQ ID NO: 16 - protein, 107 aa, Artificial Sequence
  light chain variable (VL) region
DIQMTQSPSSLSASVGDRVTITCLASQESGIWLSWYQQKPGKAPKLLIYTATSLADGVPSRFSGSGSGTDFTLTISSLQPEDFATYYCQQVYSIPWTFGGGTKVEIK

SEQ ID NO: 17 - protein, 107 aa, Artificial Sequence
  light chain variable (VL) region
DIQMTQSPSSLSASVGDRVTITCLASQTIGTWLTWYQQKPGKAPKLLIYTATSLADGVPSRFSGSGSGTDFTLTISSLQPEDFATYYCQQVAELPFGFGGGTKVEIK

SEQ ID NO: 18 - protein, 107 aa, Artificial Sequence
  light chain variable (VL) region
DIQMTQSPSSLSASVGDRVTITCLASQTIGTWLTWYQQKPGKAPKLLIYTATSLADGVPSRFSGSGSGTDFTLTISSLQPEDFATYYCQQVSVTPFTFGGGTKVEIK

SEQ ID NO: 19 - protein, 107 aa, Artificial Sequence
  light chain variable (VL) region
DIQMTQSPSSLSASVGDRVTITCLASQGIGPWLSWYQQKPGKAPKLLIYTATSLADGVPSRFSGSGSGTDFTLTISSLQPEDFATYYCQQVAELPFGFGGGTKVEIK

SEQ ID NO: 20 - protein, 107 aa, Artificial Sequence
  light chain variable (VL) region
DIQMTQSPSSLSASVGDRVTITCLASQPLGIWLSWYQQKPGKAPKLLIYTATSLADGVPSRFSGSGSGTDFTLTISSLQPEDFATYYCQQVAELPFGFGGGTKVEIK

SEQ ID NO: 21 - protein, 107 aa, Artificial Sequence
  light chain variable (VL) region
DIQMTQSPSSLSASVGDRVTITCLASQESGIWLSWYQQKPGKAPKLLIYTATSLADGVPSRFSGSGSGTDFTLTISSLQPEDFATYYCQQVAELPFGFGGGTKVEIK

SEQ ID NO: 22 - protein, 107 aa, Artificial Sequence
  light chain variable (VL) region
DIQMTQSPSSLSASVGDRVTITCLASQGIGPWLSWYQQKPGKAPKLLIYTATSLADGVPSRFSGSGSGTDFTLTISSLQPEDFATYYCQQVSVTPFTFGGGTKVEIK

SEQ ID NO: 23 - protein, 107 aa, Artificial Sequence
  light chain variable (VL) region
DIQMTQSPSSLSASVGDRVTITCLASQPLGIWLSWYQQKPGKAPKLLIYTATSLADGVPSRFSGSGSGTDFTLTISSLQPEDFATYYCQQVSVTPFTFGGGTKVEIK

SEQ ID NO: 24 - protein, 107 aa, Artificial Sequence
  light chain variable (VL) region
DIQMTQSPSSLSASVGDRVTITCLASQESGIWLSWYQQKPGKAPKLLIYTATSLADGVPSRFSGSGSGTDFTLTISSLQPEDFATYYCQQVSVTPFTFGGGTKVEIK

SEQ ID NO: 25 - protein, 327 aa, Homo sapiens
ASTKGPSVFPLAPCSRSTSESTAALGCLVKDYFPEPVTVSWNSGALTSGVHTFPAVLQSSGLYSLSSVVTVPSSSLGTKTYTCNVDHKPSNTKVDKRVESKYGPPCPSCPAPEFLGGPSVFLFPPKPKDTLMISRTPEVTCVVVDVSQEDPEVQFNWYVDGVEVHNAKTKPREEQFNSTYRVVSVLTVLHQDWLNGKEYKCKVSNKGLPSSIEKTISKAKGQPREPQVYTLPPSQEEMTKNQVSLTCLVKGFYPSDIAVEWESNGQPENNYKTTPPVLDSDGSFFLYSRLTVDKSRWQEGNVFSCSVMHEALHNHYTQKSLSLSLGK

SEQ ID NO: 26 - protein, 327 aa, Artificial Sequence
  Human IgG4(S228P) antibody Fc region
ASTKGPSVFPLAPCSRSTSESTAALGCLVKDYFPEPVTVSWNSGALTSGVHTFPAVLQSSGLYSLSSVVTVPSSSLGTKTYTCNVDHKPSNTKVDKRVESKYGPPCPPCPAPEFLGGPSVFLFPPKPKDTLMISRTPEVTCVVVDVSQEDPEVQFNWYVDGVEVHNAKTKPREEQFNSTYRVVSVLTVLHQDWLNGKEYKCKVSNKGLPSSIEKTISKAKGQPREPQVYTLPPSQEEMTKNQVSLTCLVKGFYPSDIAVEWESNGQPENNYKTTPPVLDSDGSFFLYSRLTVDKSRWQEGNVFSCSVMHEALHNHYTQKSLSLSLGK

SEQ ID NO: 27 - protein, 330 aa, Homo sapiens [sequence omitted]

SEQ ID NO: 28 - protein, 330 aa, Artificial Sequence
  Human IgG1-3M antibody Fc region
ASTKGPSVFPLAPSSKSTSGGTAALGCLVKDYFPEPVTVSWNSGALTSGVHTFPAVLQSSGLYSLSSVVTVPSSSLGTQTYICNVNHKPSNTKVDKKVEPKSCDKTHTCPPCPAPEAAGAPSVFLFPPKPKDTLMISRTPEVTCVVVDVSHEDPEVKFNWYVDGVEVHNAKTKPREEQYNSTYRVVSVLTVLHQDWLNGKEYKCKVSNKALPAPIEKTISKAKGQPREPQVYTLPPSRDELTKNQVSLTCLVKGFYPSDIAVEWESNGQPENNYKTTPPVLDSDGSFFLYSKLTVDKSRWQQGNVFSCSVMHEALHNHYTQKSLSLSPGK

SEQ ID NO: 29 - protein, 326 aa, Homo sapiens
ASTKGPSVFPLAPCSRSTSESTAALGCLVKDYFPEPVTVSWNSGALTSGVHTFPAVLQSSGLYSLSSVVTVPSSNFGTQTYTCNVDHKPSNTKVDKTVERKCCVECPPCPAPPVAGPSVFLFPPKPKDTLMISRTPEVTCVVVDVSHEDPEVQFNWYVDGVEVHNAKTKPREEQFNSTFRVVSVLTVVHQDWLNGKEYKCKVSNKGLPAPIEKTISKTKGQPREPQVYTLPPSREEMTKNQVSLTCLVKGFYPSDISVEWESNGQPENNYKTTPPMLDSDGSFFLYSKLTVDKSRWQQGNVFSCSVMHEALHNHYTQKSLSLSPGK

SEQ ID NO: 30 - protein, 330 aa, Homo sapiens
ASTKGPSVFPLAPSSKSTSGGTAALGCLVKDYFPEPVTVSWNSGALTSGVHTFPAVLQSSGLYSLSSVVTVPSSSLGTQTYICNVNHKPSNTKVDKKVEPKSCDKTHTCPPCPAPELLGGPSVFLFPPKPKDTLMISRTPEVTCVVVDVSHEDPEVKFNWYVDGVEVHNAKTKPREEQYNSTYRVVSVLTVLHQDWLNGKEYKCKVSNKALPAPIEKTISKAKGQPREPQVYTLPPSREEMTKNQVSLTCLVKGFYPSDIAVEWESNGQPENNYKTTPPVLDSDGSFFLYSKLTVDKSRWQQGNVFSCSVMHEALHNHYTQKSLSLSPGK

SEQ ID NO: 31 - protein, 329 aa, Artificial Sequence
  IgG1-3M REEM allotype antibody Fc region
ASTKGPSVFPLAPSSKSTSGGTAALGCLVKDYFPEPVTVSWNSGALTSGVHTFPAVLQSSGLYSLSSVVTVPSSSLGTQTYICNVNHKPSNTKVDKKVEPKSCDKTHTCPPCPAPEAAGAPSVFLFPPKPKDTLMISRTPEVTCVVVDVSHEDPEVKFNWYVDGVEVHNAKTKPREEQYNSTYRVVSVLTVLHQDWLNGKEYKCKVSNKALPAPIEKTISKAKGQPREPQVYTLPPSREEMKNQVSLTCLVKGFYPSDIAVEWESNGQPENNYKTTPPVLDSDGSFFLYSKLTVDKSRWQQGNVFSCSVMHEALHNHYTQKSLSLSPGK

SEQ ID NO: 32 - protein, 288 aa, Homo sapiens
MQIPQAPWPVVWAVLQLGWRPGWFLDSPDRPWNPPTFSPALLVVTEGDNATFTCSFSNTSESFVLNWYRMSPSNQTDKLAAFPEDRSQPGQDCRFRVTQLPNGRDFHMSVVRARRNDSGTYLCGAISLAPKAQIKESLRAELRVTERRAEVPTAHPSPSPRPAGQFQTLVVGVVGGLLGSLVLLVWVLAVICSRAARGTIGARRTGQPLKEDPSAVPVFSVDYGELDFQWREKTPEPPVPCVPEQTEYATIVFPSGMGTSSPARRGSADGPRSAQPLRPEDGHCSWPL

SEQ ID NO: 33 - protein, 288 aa, Macaca fascicularis
MQIPQAPWPVVWAVLQLGWRPGWFLESPDRPWNAPTFSPALLLVTEGDNATFTCSFSNASESFVLNWYRMSPSNQTDKLAAFPEDRSQPGQDCRFRVTRLPNGRDFHMSVVRARRNDSGTYLCGAISLAPKAQIKESLRAELRVTERRAEVPTAHPSPSPRPAGQFQALVVGVVGGLLGSLVLLVWVLAVICSRAAQGTIEARRTGQPLKEDPSAVPVFSVDYGELDFQWREKTPEPPAPCVPEQTEYATIVFPSGLGTSSPARRGSADGPRSPRPLRPEDGHCSWPL

SEQ ID NO: 34 - protein, 1356 aa, Homo sapiens
MQSKVLLAVALWLCVETRAASVGLPSVSLDLPRLSIQKDILTIKANTTLQITCRGQRDLDWLWPNNQSGSEQRVEVTECSDGLFCKTLTIPKVIGNDTGAYKCFYRETDLASVIYVYVQDYRSPFIASVSDQHGVVYITENKNKTVVIPCLGSISNLNVSLCARYPEKRFVPDGNRISWDSKKGFTIPSYMISYAGMVFCEAKINDESYQSIMYIVVVVGYRIYDVVLSPSHGIELSVGEKLVLNCTARTELNVGIDFNWEYPSSKHQHKKLVNRDLKTQSGSEMKKFLSTLTIDGVTRSDQGLYTCAASSGLMTKKNSTFVRVHEKPFVAFGSGMESLVEATVGERVRIPAKYLGYPPPEIKWYKNGIPLESNHTIKAGHVLTIMEVSERDTGNYTVILTNPISKEKQSHVVSLVVYVPPQIGEKSLISPVDSYQYGTTQTLTCTVYAIPPPHHIHWYWQLEEECANEPSQAVSVTNPYPCEEWRSVEDFQGGNKIEVNKNQFALIEGKNKTVSTLVIQAANVSALYKCEAVNKVGRGERVISFHVTRGPEITLQPDMQPTEQESVSLWCTADRSTFENLTWYKLGPQPLPIHVGELPTPVCKNLDTLWKLNATMFSNSTNDILIMELKNASLQDQGDYVCLAQDRKTKKRHCVVRQLTVLERVAPTITGNLENQTTSIGESIEVSCTASGNPPPQIMWFKDNETLVEDSGIVLKDGNRNLTIRRVRKEDEGLYTCQACSVLGCAKVEAFFIIEGAQEKTNLEIIILVGTAVIAMFFWLLLVIILRTVKRANGGELKTGYLSIVMDPDELPLDEHCERLPYDASKWEFPRDRLKLGKPLGRGAFGQVIEADAFGIDKTATCRTVAVKMLKEGATHSEHRALMSELKILIHIGHHLNVVNLLGACTKPGGPLMVIVEFCKFGNLSTYLRSKRNEFVPYKTKGARFRQGKDYVGAIPVDLKRRLDSITSSQSSASSGFVEEKSLSDVEEEEAPEDLYKDFLTLEHLICYSFQVAKGMEFLASRKCIHRDLAARNILLSEKNVVKICDFGLARDIYKDPDYVRKGDARLPLKWMAPETIFDRVYTIQSDVWSFGVLLWEIFSLGASPYPGVKIDEEFCRRLKEGTRMRAPDYTTPEMYQTMLDCWHGEPSQRPTFSELVEHLGNLLQANAQQDGKDYIVLPISETLSMEEDSGLSLPTSPVSCMEEEEVCDPKFHYDNTAGISQYLQNSKRKSRPVSVKTFEDIPLEEPEVKVIPDDNQTDSGMVLASEELKTLEDRTKLSPSFGGMVPSKSRESVASEGSNQTSGYQSGYHSDDTDTTVYSSEEAELLKLIEIGVQTGSTAQILQPDSGTTLSSPPV

SEQ ID NO: 35 - protein, 1356 aa, Macaca mulatta
MASKVLLAVALWLCVETRAASVGLPSVSLDLPRLSIQKDILTIKANTTLQITCRGQRDLDWLWPNNQSGSEQRVEVTECSDGLFCKTLTIPKVIGNDTGAYKCFYRETDLASVIYVYVQDYRSPFIASVSDQHGVVYITENKNKTVVIPCLGSISNLNVSLCARYPEKRFVPDGNRISWDSKKGFTIPSYMISYAGMVFCEAKINDESYQSIMYIVVVVGYRIYDVVLSPSHGVELSVGEKLVLNCTARTELNVGIDFNWEYPSSKHQHKKLVNRDLKTQSGSEMKKFLSTLTIDGVTRSDQGLYTCAASSGLMTKKNSTFVRVHEKPFVAFGSGMESLVEATVGERVRIPVKYLGYPPPEIKWYKNGIPLESNHTVKVGHVLTIMEVSERDTGNYTVILTNPISKEKQSHVVSLVVYVPPQIGEKSLISPVDSYQYGTTQTLTCTVYAIPPPHHIHWYWQLEEECPNEPSQAVSVTNPYPCEEWRSVEDFQGGNKIEVNKNQFALIEGKNKTVSTLVIQAANVSALYKCEAVNKVGRGERVISFHVTRGPEITLQPDLQPTEQESVSLWCTADKSTFENLTWYKLGPQPLPVHVGELPTPVCKNLDTLWKLNATIFSNSTNDILIMELKNASLQDQGDYVCVAQDRKTKKRHCVVRQLTVLERVAPMITGNLENQTTSIGETIEVSCTASGNPPPQIMWFKDNETLVEDSGIVLKDGNRNLTIRRVRKEDEGLYTCQACSVLGCAKVEAFFIIEGAQEKTNLEIIILVGTAVIAMFFWLLLVIILRTVKRANGGELKTGYLSIVMDPDELPLDEHCERLPYDASKWEFPRDRLKLGKPLGRGAFGQVIEADAFGIDKTATCRTVAVKMLKEGATHSEHRALMSELKILIHIGHHLNVVNLLGACTKPGGPLMVIVEFCKFGNLSTYLRSKRNEFVPYKTKGARFRQGKDYVGAIPVDLKRRLDSITSSQSSASSGFVEEKSLSDVEEEEAPEDLYKDFLTLEHLICYSFQVAKGMEFLASRKCIHRDLAARNILLSEKNVVKICDFGLARDIYKDPDYVRKGDARLPLKWMAPETIFDRVYTIQSDVWSFGVLLWEIFSLGASPYPGVKIDEEFCRRLKEGTRMRAPDYTTPEMYQTMLDCWHGEPSQRPTFSELVEHLGNLLQANAQQDGKDYIVLPISETLSMEEDSGLSLPTSPVSCMEEEEVCDPKFHYDNTAGISQYLQNSKRKSRPVSVKTFEDIPLEEPEVKVIPDDNQTDSGMVLASEELKTLEDRTKLAPSFSGMVSSKSRESVASEGSNQTSGYQSGYHSDDTDTTVYSSEEAELLKLIEIGVQTGSTAQILQPDSGTTLSSPPV

SEQ ID NO: 36 - protein, 5 aa, Unknown
  immunoglobulin constant region motif
RDELT

SEQ ID NO: 37 - protein, 4 aa, Unknown
  immunoglobulin constant region motif
REEM

SEQ ID NO: 38 - protein, 17 aa, Artificial Sequence
  VH HCDR2
TISGGGANTYYVDSVKG

SEQ ID NO: 39 - protein, 11 aa, Artificial Sequence
  VL LCDR1
RASQESGIWLS

SEQ ID NO: 40 - protein, 7 aa, Artificial Sequence
  VL LCDR2
TASSLAD

SEQ ID NO: 41 - protein, 7 aa, Artificial Sequence
  VL LCDR2
AASSLAD

SEQ ID NO: 42 - protein, 17 aa, Artificial Sequence
  VH HCDR2
TISGGGSNKYYVDSVKG

SEQ ID NO: 43 - protein, 7 aa, Artificial Sequence
  VL LCDR2
AASSLQS

SEQ ID NO: 44 - protein, 107 aa, Artificial Sequence
  light chain variable (VL) region
DIQMTQSPSSLSASVGDRVTITCRASQESGIWLSWYQQKPGKAPKLLIYTATSLADGVPSRFSGSGSGTDFTLTISSLQPEDFATYYCQQVSVTPFTFGGGTKVEIK

SEQ ID NO: 45 - protein, 107 aa, Artificial Sequence
  light chain variable (VL) region
DIQMTQSPSSLSASVGDRVTITCRASQESGIWLSWYQQKPGKAPKLLIYTASSLADGVPSRFSGSGSGTDFTLTISSLQPEDFATYYCQQVSVTPFTFGGGTKVEIK

SEQ ID NO: 46 - protein, 107 aa, Artificial Sequence
  light chain variable (VL) region
DIQMTQSPSSLSASVGDRVTITCRASQESGIWLSWYQQKPGKAPKLLIYAASSLADGVPSRFSGSGSGTDFTLTISSLQPEDFATYYCQQVSVTPFTFGGGTKVEIK

SEQ ID NO: 47 - protein, 107 aa, Artificial Sequence
  light chain variable (VL) region
DIQMTQSPSSLSASVGDRVTITCRASQESGIWLSWYQQKPGKAPKLLIYAASSLQSGVPSRFSGSGSGTDFTLTISSLQPEDFATYYCQQVSVTPFTFGGGTKVEIK

SEQ ID NO: 48 - protein, 116 aa, Artificial Sequence
  heavy chain variable (VH) region
EVQLVESGGGLVQPGGSLRLSCAASGFTFSSYMMSWVRQAPGKGLEWVATISGGGANTYYVDSVKGRFTISRDNAKNSLYLQMNSLRAEDTAVYYCARQLYYFDYWGQGTTVTVSS

SEQ ID NO: 49 - protein, 116 aa, Artificial Sequence
  heavy chain variable (VH) region
EVQLVESGGGLVQPGGSLRLSCAASGFTFSSYMMSWVRQAPGKGLEWVATISGGGSNKYYVDSVKGRFTISRDNAKNSLYLQMNSLRAEDTAVYYCARQLYYFDYWGQGTTVTVSS

SEQ ID NO: 50 - protein, 23 aa, Artificial Sequence
  VL LFR1
DIQMTQSPSSLSASVGDRVTITC

SEQ ID NO: 51 - protein, 15 aa, Artificial Sequence
  VL LFR2
WYQQKPGKAPKLLIY

SEQ ID NO: 52 - protein, 32 aa, Artificial Sequence
  VL LFR3
GVPSRFSGSGSGTDFTLTISSLQPEDFATYYC

SEQ ID NO: 53 - protein, 10 aa, Artificial Sequence
  VL LFR4
FGGGTKVEIK

SEQ ID NO: 54 - protein, 25 aa, Artificial Sequence [sequence omitted]

SEQ ID NO: 55 - protein, 12 aa, Artificial Sequence
  VH HFR2
WVRQAPGKGLEW

SEQ ID NO: 56 - protein, 19 aa, Artificial Sequence
  VH HCDR2
VATISGGGANTYYPDSVKG

SEQ ID NO: 57 - protein, 32 aa, Artificial Sequence
  VH HFR3
RFTISRDNAKNSLYLQMNSLRAEDTAVYYCAR

SEQ ID NO: 58 - protein, 11 aa, Artificial Sequence
  VH HFR4
WGQGTTVTVSS

SEQ ID NO: 59 - protein, 11 aa, Artificial Sequence
  VL LCDR1
  MISC_FEATURE (5)..(5): Xaa is Thr, Glu, Gly, Lys, Pro or Ser
  MISC_FEATURE (6)..(6): Xaa is Ile, Ala, Leu, Ser or Val
  MISC_FEATURE (7)..(7): Xaa is Gly, Arg or Ser
  MISC_FEATURE (8)..(8): Xaa is Thr, Gly, Ile, Leu or Pro
  MISC_FEATURE (11)..(11): Xaa is Thr or Ser
LASQXXXXWLX

SEQ ID NO: 60 - protein, 9 aa, Artificial Sequence
  VL LCDR3
  MISC_FEATURE (4)..(4): Xaa is Tyr, Ala, Phe, Asn or Ser
  MISC_FEATURE (5)..(5): Xaa is Ser, Ala, Glu, Met, Asn, Gln or Val
  MISC_FEATURE (6)..(6): Xaa is Ile, Leu, Thr or Val
  MISC_FEATURE (8)..(8): Xaa is Trp or Phe
  MISC_FEATURE (9)..(9): Xaa is Thr, Ala, Gly, Asn, Arg or Ser
QQVXXXPXX

SEQ ID NO: 61 - protein, 10 aa, Artificial Sequence
  VH HCDR1
GFTFSSYLMS

SEQ ID NO: 62 - protein, 7 aa, Artificial Sequence
  VH HCDR3
QLYFFDY

SEQ ID NO: 63 - protein, 7 aa, Artificial Sequence
  VH HCDR3
QLYYYDY

SEQ ID NO: 64 - protein, 7 aa, Artificial Sequence
  VH HCDR3
QVYYFDY

SEQ ID NO: 65 - protein, 7 aa, Artificial Sequence
  VH HCDR3
QLYGFDY

SEQ ID NO: 66 - protein, 7 aa, Artificial Sequence
  VH HCDR3
QLYYADY

SEQ ID NO: 67 - protein, 116 aa, Artificial Sequence
  heavy chain variable (VH) region
EVQLVESGGGLVQPGGSLRLSCAASGFTFSSYLMSWVRQAPGKGLEWVATISGGGSNKYYVDSVKGRFTISRDNAKNSLYLQMNSLRAEDTAVYYCARQLYYFDYWGQGTTVTVSS

SEQ ID NO: 68 - protein, 116 aa, Artificial Sequence
  heavy chain variable (VH) region
EVQLVESGGGLVQPGGSLRLSCAASGFTFSSYLMSWVRQAPGKGLEWVATISGGGSNKYYVDSVKGRFTISRDNAKNSLYLQMNSLRAEDTAVYYCARQVYYFDYWGQGTTVTVSS

SEQ ID NO: 69 - protein, 116 aa, Artificial Sequence
  heavy chain variable (VH) region
EVQLVESGGGLVQPGGSLRLSCAASGFTFSSYLMSWVRQAPGKGLEWVATISGGGSNKYYVDSVKGRFTISRDNAKNSLYLQMNSLRAEDTAVYYCARQLYGFDYWGQGTTVTVSS

SEQ ID NO: 70 - protein, 116 aa, Artificial Sequence
  heavy chain variable (VH) region
EVQLVESGGGLVQPGGSLRLSCAASGFTFSSYLMSWVRQAPGKGLEWVATISGGGSNKYYVDSVKGRFTISRDNAKNSLYLQMNSLRAEDTAVYYCARQLYYADYWGQGTTVTVSS

SEQ ID NO: 71 - protein, 116 aa, Artificial Sequence
  heavy chain variable (VH) region
EVQLVESGGGLVQPGGSLRLSCAASGFTFSSYLMSWVRQAPGKGLEWVATISGGGSNKYYVDSVKGRFTISRDNAKNSLYLQMNSLRAEDTAVYYCARQLYFFDYWGQGTTVTVSS

SEQ ID NO: 72 - protein, 116 aa, Artificial Sequence
  heavy chain variable (VH) region
EVQLVESGGGLVQPGGSLRLSCAASGFTFSSYLMSWVRQAPGKGLEWVATISGGGSNKYYVDSVKGRFTISRDNAKNSLYLQMNSLRAEDTAVYYCARQLYYYDYWGQGTTVTVSS

SEQ ID NO: 73 - protein, 116 aa, Artificial Sequence
  heavy chain variable (VH) region
EVQLVESGGGLVQPGGSLRLSCAASGFTFSSYMMSWVRQAPGKGLEWVATISGGGSNKYYVDSVKGRFTISRDNAKNSLYLQMNSLRAEDTAVYYCARQVYYFDYWGQGTTVTVSS

SEQ ID NO: 74 - protein, 116 aa, Artificial Sequence
  heavy chain variable (VH) region
EVQLVESGGGLVQPGGSLRLSCAASGFTFSSYMMSWVRQAPGKGLEWVATISGGGSNKYYVDSVKGRFTISRDNAKNSLYLQMNSLRAEDTAVYYCARQLYYADYWGQGTTVTVSS

SEQ ID NO: 75 - protein, 116 aa, Artificial Sequence
  heavy chain variable (VH) region
EVQLVESGGGLVQPGGSLRLSCAASGFTFSSYMMSWVRQAPGKGLEWVATISGGGSNKYYVDSVKGRFTISRDNAKNSLYLQMNSLRAEDTAVYYCARQLYYYDYWGQGTTVTVSS